European Patent Specification EP 3 476 862 B1, published January 1, 2025. Title: HUMAN ANTIBODIES SPECIFICALLY BINDING TO ACNE USING PHAGE DISPLAY TECHNOLOGIES AND USES THEREOF. Applicant: E&S Healthcare Co., Ltd. The sequence listing filed with the application follows.

SEQUENCE LISTING (32 sequences)

SEQ ID NO: 1 - protein, 8 aa, Artificial Sequence
  CDRH1 OF 3F ANTIBODY
GYTFTDYY

SEQ ID NO: 2 - protein, 8 aa, Artificial Sequence
  CDRH2 OF 3F ANTIBODY
INPNSGAP

SEQ ID NO: 3 - protein, 15 aa, Artificial Sequence
  CDRH3 OF 3F ANTIBODY
VKGLEHAAGSAIFDR

SEQ ID NO: 4 - protein, 9 aa, Artificial Sequence
  CDRL1 OF 3F ANTIBODY
SGSVSTSHF

SEQ ID NO: 5 - protein, 3 aa, Artificial Sequence
  CDRL2 OF 3F ANTIBODY
FKD

SEQ ID NO: 6 - protein, 10 aa, Artificial Sequence
  CDRL3 OF 3F ANTIBODY
ALSMGSGIWV

SEQ ID NO: 7 - protein, 8 aa, Artificial Sequence
  CDRH1 OF 6F ANTIBODY
GFTFDDHG

SEQ ID NO: 8 - protein, 8 aa, Artificial Sequence
  CDRH2 OF 6F ANTIBODY
INLNGGST

SEQ ID NO: 9 - protein, 7 aa, Artificial Sequence
  CDRH3 OF 6F ANTIBODY
STRHLHH

SEQ ID NO: 10 - protein, 11 aa, Artificial Sequence
  CDRL1 OF 6F ANTIBODY
QSLVHSNGNTY

SEQ ID NO: 11 - protein, 3 aa, Artificial Sequence
  CDRL2 OF 6F ANTIBODY
KIS

SEQ ID NO: 12 - protein, 9 aa, Artificial Sequence
  CDRL3 OF 6F ANTIBODY
VQAKQFPLT

SEQ ID NO: 13 - protein, 8 aa, Artificial Sequence
  CDRH1 OF 8F ANTIBODY
GFSFNDYA

SEQ ID NO: 14 - protein, 8 aa, Artificial Sequence
  CDRH2 OF 8F ANTIBODY
ISWNSRST

SEQ ID NO: 15 - protein, 16 aa, Artificial Sequence
  CDRH3 OF 8F ANTIBODY
TTDLGVVPAAIYAFDI

SEQ ID NO: 16 - protein, 6 aa, Artificial Sequence
  CDRL1 OF 8F ANTIBODY
QGITNW

SEQ ID NO: 17 - protein, 3 aa, Artificial Sequence
  CDRL2 OF 8F ANTIBODY
AAS

SEQ ID NO: 18 - protein, 9 aa, Artificial Sequence
  CDRL3 OF 8F ANTIBODY
QQTATFQIT

SEQ ID NO: 19 - protein, 8 aa, Artificial Sequence
  CDRH1 OF 10F ANTIBODY
GFTVSSSF

SEQ ID NO: 20 - protein, 7 aa, Artificial Sequence
  CDRH2 OF 10F ANTIBODY
AYSGGNT

SEQ ID NO: 21 - protein, 17 aa, Artificial Sequence
  CDRH3 OF 10F ANTIBODY
SCEGKAVSGSRDLHFEF

SEQ ID NO: 22 - protein, 6 aa, Artificial Sequence
  CDRL1 OF 10F ANTIBODY
NLRTKY

SEQ ID NO: 23 - protein, 3 aa, Artificial Sequence
  CDRL2 OF 10F ANTIBODY
NDN

SEQ ID NO: 24 - protein, 11 aa, Artificial Sequence
  CDRL3 OF 10F ANTIBODY
QVWDSSSDHLI

SEQ ID NO: 25 - protein, 122 aa, Artificial Sequence
  3F HEAVY CHAIN VARIABLE REGION(VH)
QMQLVQSGAEVKKPGASVKVSCKASGYTFTDYYIHWVRQAPGQGLEWMGWINPNSGAPEFAQRFQGRVSMTRDASINTTYMELSGLRSEDTAVYYCVKGLEHAAGSAIFDRWGQGTMVTVSS

SEQ ID NO: 26 - protein, 110 aa, Artificial Sequence
  3F LIGHT CHAIN VARIABLE REGION(VL)
QTVVTQEPSFSVSPGGTVTLTCGLTSGSVSTSHFPSWYQQTPGQAPRTLIYFKDTRSSGVPDRFSGSILGNKAALTITGAQADDESDYYCALSMGSGIWVFGGGTKLTVL

SEQ ID NO: 27 - protein, 114 aa, Artificial Sequence
  6F HEAVY CHAIN VARIABLE REGION(VH)
QVQLVESGGGVVRPGGSLRLSCTASGFTFDDHGMSWVRQAPGKGLEWVSTINLNGGSTAYADSVKGRFTISRDNAKNSLYLQMNSLRAEDTAVYYCSTRHLHHWGQGTLVTVSS

SEQ ID NO: 28 - protein, 112 aa, Artificial Sequence
  6F LIGHT CHAIN VARIABLE REGION(VL)
DIVMTQTPLSSPVTLGQPASISCRSSQSLVHSNGNTYLTWLQQRPGQPPRLLIHKISNRFSGVPDRFSGSGAGTDFTLKISRVEAEDVGVYYCVQAKQFPLTFGQGTRLEIK

SEQ ID NO: 29 - protein, 123 aa, Artificial Sequence
  8F HEAVY CHAIN VARIABLE REGION(VH)
QVQLVQSGGGVVQPGGSLRLSCAASGFSFNDYAMHWVRQVPGKGLEWVSSISWNSRSTVYAASVEGRFSISRDNSKNSLYLQMNSLRAEDAAVYYCTTDLGVVPAAIYAFDIWGQGTMVTVSS

SEQ ID NO: 30 - protein, 107 aa, Artificial Sequence
  8F LIGHT CHAIN VARIABLE REGION(VL)
DIQMTQSPSVMSASVGDRVNITCRASQGITNWLAWYQQKPGKAPKLLISAASSLQSGVPSRFSGSGSGTDFTLTISSLQPDDFATYYCQQTATFQITFGQGTRLDIK

SEQ ID NO: 31 - protein, 123 aa, Artificial Sequence
  10F HEAVY CHAIN VARIABLE REGION(VH)
QVQLVESGGGLIQPGGSLRLSCVASGFTVSSSFMSWVRLAPGKGLEWVALAYSGGNTYYADSVKGRFTVSRDDSSNTLYLQMNSLRAEDTAVYYCSCEGKAVSGSRDLHFEFWSPGTLVTVSS

SEQ ID NO: 32 - protein, 108 aa, Artificial Sequence
  10F LIGHT CHAIN VARIABLE REGION(VL)
SYELTQAPSLSVSPGQTANIICSGDNLRTKYVSWYQQKPGQAPVLVIYNDNDRPSGIPERFSGTNSGNTAALTISRVEAGDEADYYCQVWDSSSDHLIFGGGTKLTVL